European Patent Specification EP 4 043 076 B1, published June 26, 2024. Title: Cyclic peptide having CTLA-4-Inhibiting Activity and Use Thereof. Applicant: GeneFrontier. The sequence listing filed with the application follows.

SEQUENCE LISTING (211 sequences)

SEQ ID NO: 1 - protein, 223 aa, Homo sapiens
MACLGFQRHKAQLNLATRTWPCTLLFFLLFIPVFCKAMHVAQPAVVLASSRGIASFVCEYASPGKATEVRVTVLRQADSQVTEVCAATYMMGNELTFLDDSICTGTSSGNQVNLTIQGLRAMDTGLYICKVELMYPPPYYLGIGNGTQIYVIDPEPCPDSDFLLWILAAVSSGLFFYSFLLTAVSLSKMLKKRSPLTTGVYVKMPPTEPECEKQFQPYFIPIN

SEQ ID NO: 2 - protein, 288 aa, Homo sapiens
MGHTRRQGTSPSKCPYLNFFQLLVLAGLSHFCSGVIHVTKEVKEVATLSCGHNVSVEELAQTRIYWQKEKKMVLTMMSGDMNIWPEYKNRTIFDITNNLSIVILALRPSDEGTYECVVLKYEKDAFKREHLAEVTLSVKADFPTPSISDFEIPTSNIRRIICSTSGGFPEPHLSWLENGEELNAINTTVSQDPETELYAVSSKLDFNMTTNHSFMCLIKYGHLRVNQTFNWNTTKQEHFPDNLLPSWAITLISVNGIFVICCLTYCFAPRCRERRRNERLRRESVRPV

SEQ ID NO: 3 - DNA, 108 bp, Artificial Sequence
  Oligo DNA encoding randomized amino acid sequence
  misc_feature (34)..(35): n is a, c, g, or t
  misc_feature (37)..(38): n is a, c, g, or t
  misc_feature (40)..(41): n is a, c, g, or t
  misc_feature (43)..(44): n is a, c, g, or t
  misc_feature (46)..(47): n is a, c, g, or t
  misc_feature (49)..(50): n is a, c, g, or t
  misc_feature (52)..(53): n is a, c, g, or t
  misc_feature (55)..(56): n is a, c, g, or t
  misc_feature (58)..(59): n is a, c, g, or t
  misc_feature (61)..(62): n is a, c, g, or t
  misc_feature (64)..(65): n is a, c, g, or t
  misc_feature (67)..(68): n is a, c, g, or t
gactataaagatgacgatgacaaaggcgggtgcnnsnnsnnsnnsnnsnnsnnsnnsnnsnnsnnsnnstgtggaggcgagcagaagctgatctctgaggaggatctg

SEQ ID NO: 4 - protein, 36 aa, Artificial Sequence
  cyclic peptide with randomized amino acid sequence
  misc_feature (12)..(23): Xaa can be any naturally occurring amino acid
DYKDDDDKGGCXXXXXXXXXXXXCGGEQKLISEEDL

SEQ ID NO: 5 - DNA, 112 bp, Artificial Sequence
  5'UTR Oligo DNA
gaaattaatacgactcactatagggagaccacaacggtttccctctagaaataattttgtttaactttaagaaggagatataccaatggactataaagatgacgatgacaaa

SEQ ID NO: 6 - DNA, 60 bp, Artificial Sequence
  Primer Myc-g3p
gagcagaagctgatctctgaggaggatctgaagcttgaatatcaaggccaatcgtctgac

SEQ ID NO: 7 - DNA, 108 bp, Artificial Sequence
  Primer g3p-SecMstop
ctcgagttattcattaggtgaggcgttgagggccagcacggatgccttgcgcctggcttatccagacgggcgtgctgaattttgcgccggaaacgtcaccaatgaaac

SEQ ID NO: 8 - DNA, 48 bp, Artificial Sequence
  5' primer
gaaattaatacgactcactatagggagaccacaacggtttccctctag

SEQ ID NO: 9 - DNA, 32 bp, Artificial Sequence
  Primer SecMstop
ggattagttattcattaggtgaggcgttgagg

SEQ ID NO: 10 - DNA, 22 bp, Artificial Sequence
  RT reverse primer Myc R
cagatcctcctcagagatcagc

SEQ ID NO: 11 - DNA, 29 bp, Artificial Sequence
  Primer FLAG F
atggactataaagatgacgatgacaaagg

SEQ ID NO: 12 - DNA, 35 bp, Artificial Sequence
  Primer Eco1-(-M)-FLAG_F
ccgaattcgactataaagatgacgatgacaaaggc

SEQ ID NO: 13 - DNA, 33 bp, Artificial Sequence
  Primer Myc-Hind3_R
aaaaaaaaaagcttcagatcctcctcagagatc

SEQ ID NO: 14 - DNA, 28 bp, Artificial Sequence
  Primer pET-MALseqF
ccagaaaggtgaaatcatgccgaacatc

SEQ ID NO: 15 - protein, 14 aa, Artificial Sequence
  H12SSI-Ctla4-3-02
CMHPFLLVVSHHFC

SEQ ID NO: 16 - protein, 14 aa, Artificial Sequence
  H12SSI-Ctla4-3-51
CGLGQGYWFKVWFC

SEQ ID NO: 17 - protein, 14 aa, Artificial Sequence
  H12SSI-Ctla4-3-33
CAKNFGYWYHQWFC

SEQ ID NO: 18 - protein, 14 aa, Artificial Sequence
  H12SSI-Ctla4-3-80
CGAGKGFWFKVWFC

SEQ ID NO: 19 - protein, 14 aa, Artificial Sequence
  H12SSI-Ctla4-2-23
CGFHDGFWYNVWFC

SEQ ID NO: 20 - protein, 14 aa, Artificial Sequence
  H12SSI-Ctla4-3-90
CGVNLGFWFNVWFC

SEQ ID NO: 21 - protein, 14 aa, Artificial Sequence
  H12SSI-Ctla4-3-38
CIIQGQYWWNIWHC

SEQ ID NO: 22 - protein, 16 aa, Artificial Sequence
  Clone #19
CMHPFLPIVSHHFCER

SEQ ID NO: 23 - protein, 15 aa, Artificial Sequence
  Original clone
KCMHPFLLVVSHHFC

SEQ ID NO: 24 - protein, 17 aa, Artificial Sequence
  Clone #19
KCMHPFLPIVSHHFCER

SEQ ID NO: 25 - protein, 15 aa, Artificial Sequence
  Original clone
GCMHPFLLVVSHHFC

SEQ ID NO: 26 - protein, 17 aa, Artificial Sequence
  Clone #19
GCMHPFLPIVSHHFCER

SEQ ID NO: 27 - protein, 16 aa, Artificial Sequence
  Clone #10
CLHPFLPIVSHHFCGR

SEQ ID NO: 28 - DNA, 114 bp, Artificial Sequence
  Randomized oligo DNA
  misc_feature (34)..(35): n is a, c, g, or t
  misc_feature (43)..(44): n is a, c, g, or t
  misc_feature (55)..(56): n is a, c, g, or t
  misc_feature (61)..(62): n is a, c, g, or t
  misc_feature (73)..(74): n is a, c, g, or t
  misc_feature (76)..(77): n is a, c, g, or t
gactataaagatgacgatgacaaaggcggttgcnnscatccannsctgccgatannstcannscatttctgtnnsnnsggatccgagcagaagctgatctctgaggaggatctg

SEQ ID NO: 29 - protein, 18 aa, Artificial Sequence
  Original clone
GGCMHPFLLVVSHHFCGG

SEQ ID NO: 30 - protein, 18 aa, Artificial Sequence
  C4-302mat-1-1-24
GGCMHPFLPVVSHHFCGG

SEQ ID NO: 31 - protein, 18 aa, Artificial Sequence
  C4-302mat-2-100-18
GGCMHPFLPVVSHHFCRG

SEQ ID NO: 32 - protein, 18 aa, Artificial Sequence
  C4-302mat-3-1-48
GGCMHPFLPVVSHHFCGA

SEQ ID NO: 33 - protein, 18 aa, Artificial Sequence
  C4-302mat-3-100-37
GGCMHPFLPVVSHHFCGR

SEQ ID NO: 34 - protein, 18 aa, Artificial Sequence
  C4-302mat-1-1-35
GGCMHPFLPVASHHFCGG

SEQ ID NO: 35 - protein, 18 aa, Artificial Sequence
  C4-302mat-3-1-22
GGCMHPFLPVASHHFCGR

SEQ ID NO: 36 - protein, 18 aa, Artificial Sequence
  C4-302mat-3-100-27
GGCMHPFLPVASHHFCAG

SEQ ID NO: 37 - protein, 18 aa, Artificial Sequence
  GGCLHPFLPVVSHHFCGD
GGCLHPFLPVVSHHFCGD

SEQ ID NO: 38 - protein, 18 aa, Artificial Sequence
  C4-302mat-2-1-38
GGCLHPFLPLVSHHFCGG

SEQ ID NO: 39 - protein, 18 aa, Artificial Sequence
  C4-302mat-3-100-44
GGCLHPFLPIVSHHFCGR

SEQ ID NO: 40 - protein, 18 aa, Artificial Sequence
  C4-302mat-3-1-45
GGCRHPFLPIVSRHFCRG

SEQ ID NO: 41 - protein, 18 aa, Artificial Sequence
  C4-302mat-3-100-20
GGCVHPFLPVVSHHFCRG

SEQ ID NO: 42 - protein, 18 aa, Artificial Sequence
  C4-302mat-3-100-9
GGCKHPFLPVVSHHFCGG

SEQ ID NO: 43 - protein, 18 aa, Artificial Sequence
  C4-302mat-3-1-10
GGCKHPYLPVASHHFCRG

SEQ ID NO: 44 - protein, 18 aa, Artificial Sequence
  C4-302mat-2-1-27
GGCMHPYLPVISHHFCGG

SEQ ID NO: 45 - protein, 18 aa, Artificial Sequence
  C4-302mat-3-100-12
GGCMHPYLPVISHHFCGR

SEQ ID NO: 46 - protein, 18 aa, Artificial Sequence
  C4-302mat-2-1-3
GGCMHPFLPVTSHHFCGG

SEQ ID NO: 47 - protein, 18 aa, Artificial Sequence
  C4-302mat-2-100-27
GGCMHPFLPIVSHHFCGS

SEQ ID NO: 48 - protein, 18 aa, Artificial Sequence
  C4-302mat-3-1-27
GGCMHPFLPIVSHHFCER

SEQ ID NO: 49 - protein, 18 aa, Artificial Sequence
  C4-302mat-3-1-23
GGCMHPFLPIASLHFCGR

SEQ ID NO: 50 - protein, 18 aa, Artificial Sequence
  C4-302mat-3-1-32
GGCMHPFLPILSHHFCAG

SEQ ID NO: 51 - protein, 18 aa, Artificial Sequence
  C4-302mat-3-1-31
GSCMHPFLPVASRHFCGR

SEQ ID NO: 52 - protein, 18 aa, Artificial Sequence
  C4-302mat-3-1-5
GGCMHPFLPVVSRHFCGG

SEQ ID NO: 53 - protein, 18 aa, Artificial Sequence
  C4-302mat-3-1-12
GGCMHPFLPVVSRHFCGR

SEQ ID NO: 54 - protein, 18 aa, Artificial Sequence
  C4-302mat-3-1-35
GGCMHPFLQTVSHHFCGG

SEQ ID NO: 55 - protein, 18 aa, Artificial Sequence
  C4-302mat-2-1-35
GGCMHPFLQVVSHHFCGS

SEQ ID NO: 56 - protein, 18 aa, Artificial Sequence
  C4-302mat-2-100-4
GGCMHPFLQVVSHHFCGG

SEQ ID NO: 57 - protein, 18 aa, Artificial Sequence
  C4-302mat-1-1-21
GGCIHPFLQVVSHHFCGG

SEQ ID NO: 58 - protein, 18 aa, Artificial Sequence
  C4-302mat-1-100-23
GGCVHPFLQVVSHHFCGG

SEQ ID NO: 59 - protein, 18 aa, Artificial Sequence
  C4-302mat-2-1-40
GGCMHPFLQVASHHFCGG

SEQ ID NO: 60 - protein, 18 aa, Artificial Sequence
  C4-302mat-3-1-2
GGCMHPYLQVVSHHFCGR

SEQ ID NO: 61 - protein, 18 aa, Artificial Sequence
  C4-302mat-1-1-37
GGCMHPFLRVVSHHFCGG

SEQ ID NO: 62 - protein, 18 aa, Artificial Sequence
  C4-302mat-3-1-14
GGCMHPFLRVVSHHFCGR

SEQ ID NO: 63 - protein, 18 aa, Artificial Sequence
  C4-302mat-2-1-12
GGCKHPFLRVVSHHFCRR

SEQ ID NO: 64 - protein, 18 aa, Artificial Sequence
  C4-302mat-2-1-24
GGCMHPFLRIVSQHFCRR

SEQ ID NO: 65 - protein, 18 aa, Artificial Sequence
  C4-302mat-3-1-8
GGCMHPFLKIASHHFCGG

SEQ ID NO: 66 - protein, 18 aa, Artificial Sequence
  C4-302mat-2-1-37
GGCMHPFLLVASHHFCGV

SEQ ID NO: 67 - protein, 18 aa, Artificial Sequence
  C4-302mat-2-100-33
GSCMHPFLLVASHHFCRG

SEQ ID NO: 68 - protein, 18 aa, Artificial Sequence
  C4-302mat-3-1-9
GGCMHPYLLVASHHFCER

SEQ ID NO: 69 - protein, 18 aa, Artificial Sequence
  C4-302mat-2-100-24
GGCMHPYLLVVSHHFCGR

SEQ ID NO: 70 - protein, 18 aa, Artificial Sequence
  C4-302mat-3-1-15
GGCMHPYLLVVSRHFCGR

SEQ ID NO: 71 - protein, 18 aa, Artificial Sequence
  C4-302mat-3-1-25
GDCKHPYLLTVSHHFCGR

SEQ ID NO: 72 - protein, 18 aa, Artificial Sequence
  C4-302mat-2-100-40
GGCMHPFLLVVSRHFCGR

SEQ ID NO: 73 - protein, 18 aa, Artificial Sequence
  C4-302mat-3-1-11
GGCMHPFLLTVSRHFCGG

SEQ ID NO: 74 - protein, 18 aa, Artificial Sequence
  C4-302mat-3-100-39
GGCKHPFLLIVSHHFCGR

SEQ ID NO: 75 - protein, 18 aa, Artificial Sequence
  C4m#19-5th4w-NN6-67
GGCLHPFLPIRSVHFCPR

SEQ ID NO: 76 - protein, 18 aa, Artificial Sequence
  GGCLHPFLPIRSVHFCPF
GGCLHPFLPIRSVHFCPF

SEQ ID NO: 77 - protein, 18 aa, Artificial Sequence
  C4m#19-5th4w-NN6-25
GGCLHPVLPIRSRHFCPV

SEQ ID NO: 78 - protein, 18 aa, Artificial Sequence
  C4m#19-5th4w-NN6-21
GGCWHPWLPILSPHFCPR

SEQ ID NO: 79 - protein, 18 aa, Artificial Sequence
  C4m#19-5th4w-NN6-39
GGCWHPFLPIRSLHFCPR

SEQ ID NO: 80 - protein, 18 aa, Artificial Sequence
  C4m#19-5th4w-NN6-70
GGCMHPFLPIRSMHFCPL

SEQ ID NO: 81 - protein, 18 aa, Artificial Sequence
  C4m#19-5th2w-NNS6-14
GGCWHPFLPIRSYHFCPW

SEQ ID NO: 82 - protein, 18 aa, Artificial Sequence
  C4m#19-5th4w-NN6-47
GGCPHPWLPIFSRHFCPV

SEQ ID NO: 83 - protein, 18 aa, Artificial Sequence
  C4m#19-5th4w-NN6-54
GGCLHPGLPIRSLHFCPR

SEQ ID NO: 84 - protein, 18 aa, Artificial Sequence
  C4m#19-5th4w-NN6-81
GGCFHPYLPIRSWHFCSR

SEQ ID NO: 85 - protein, 18 aa, Artificial Sequence
  C4m#19-5th4w-NN6-53
GGCRHPFLPIYSVHFCAC

SEQ ID NO: 86 - protein, 18 aa, Artificial Sequence
  C4m#19-5th4w-NN6-34
GGCFHPFLPIRSDHFCSR

SEQ ID NO: 87 - protein, 18 aa, Artificial Sequence
  C4m#19-5th4w-NN6-4
GGCRHPYLPIVSRHFCPF

SEQ ID NO: 88 - protein, 18 aa, Artificial Sequence
  C4m#19-5th2w-NNS6-21
GGCWHPFLPIRSSHFCPS

SEQ ID NO: 89 - protein, 18 aa, Artificial Sequence
  C4m#19-5th4w-NN6-20
GGCSHPQLPILSDHFCSA

SEQ ID NO: 90 - protein, 18 aa, Artificial Sequence
  C4m#19-5th4w-NN6-77
GGCRHPFLPIVSTHFCSR

SEQ ID NO: 91 - protein, 18 aa, Artificial Sequence
  C4m#19-5th4w-NN6-23
GGCRHPHLPIWSWHFCGR

SEQ ID NO: 92 - protein, 18 aa, Artificial Sequence
  C4m#19-5th4w-NN6-44
GGCRHPFLPIVSWHFCGR

SEQ ID NO: 93 - protein, 18 aa, Artificial Sequence
  C4m#19-5th4w-NN6-92-1
GGCVHPFLPIRSVHFCAL

SEQ ID NO: 94 - protein, 18 aa, Artificial Sequence
  C4m#19-5th4w-NN6-91
GGCMHPYLRIISPHFCRG

SEQ ID NO: 95 - protein, 18 aa, Artificial Sequence
  C4m#19-5th4w-NN6-19
GGCRHPYLPIWSIHFCQK

SEQ ID NO: 96 - protein, 18 aa, Artificial Sequence
  C4m#19-5th4w-NN6-55-1
GGCWHPFLPISSPHFCGR

SEQ ID NO: 97 - protein, 18 aa, Artificial Sequence
  C4m#19-5th4w-NN6-55-4
GGCVHPSLPILSVHFCPR

SEQ ID NO: 98 - protein, 18 aa, Artificial Sequence
  C4m#19-5th2w-NNS6-22
GGCMHPFLPIQSVHFCSR

SEQ ID NO: 99 - protein, 18 aa, Artificial Sequence
  C4m#19-5th4w-NN6-93
GGCCHPWLPIVSTHFCGL

SEQ ID NO: 100 - protein, 18 aa, Artificial Sequence
  C4m#19-5th4w-NN6-9
GGCFHPYLPIRSWHFCGR

SEQ ID NO: 101 - protein, 18 aa, Artificial Sequence
  C4m#19-5th4w-NN6-52
GGCLHPFLPIRSVHFCGC

SEQ ID NO: 102 - protein, 18 aa, Artificial Sequence
  C4m#19-5th2w-NNS6-55
GGCMHPYLPIKSVHFCPL

SEQ ID NO: 103 - protein, 18 aa, Artificial Sequence
  C4m#19-5th4w-NN6-82
GGCFHPFLPIRSLHFCCR

SEQ ID NO: 104 - protein, 18 aa, Artificial Sequence
  C4m#19-5th4w-NN6-50
GGCKHPVLPIWSWHFCRI

SEQ ID NO: 105 - protein, 18 aa, Artificial Sequence
  C4m#19-5th4w-NN6-78
GGCWHPALPIRSWHFCPR

SEQ ID NO: 106 - protein, 18 aa, Artificial Sequence
  C4m#19-5th4w-NN6-57
GGCMHPYLPIVSVHFCPC

SEQ ID NO: 107 - protein, 18 aa, Artificial Sequence
  C4m#19-5th4w-NN6-59
GGCLHPHLPIWSLHFCPL

SEQ ID NO: 108 - protein, 18 aa, Artificial Sequence
  C4m#19-5th4w-NN6-24
GGCWHPWLPIYSHHFCPI

SEQ ID NO: 109 - protein, 18 aa, Artificial Sequence
  C4m#19-5th4w-NN6-32
GGCPHPFLPIWSVHFCPF

SEQ ID NO: 110 - protein, 18 aa, Artificial Sequence
  C4m#19-5th4w-NN6-56
GGCWHPFLPIQSLHFCGV

SEQ ID NO: 111 - protein, 18 aa, Artificial Sequence
  C4m#19-5th2w-NNS6-67
GGCQHPWLPISSWHFCPR

SEQ ID NO: 112 - protein, 18 aa, Artificial Sequence
  C4m#19-5th4w-NN6-69-1
GGCSHPFLPILSVHFCPF

SEQ ID NO: 113 - protein, 18 aa, Artificial Sequence
  C4m#19-5th4w-NN6-69-3
GGCLHPWLPIVSVHFCAR

SEQ ID NO: 114 - protein, 18 aa, Artificial Sequence
  C4m#19-5th4w-NN6-79
GGCWHPVLPIRSCHFCAV

SEQ ID NO: 115 - protein, 18 aa, Artificial Sequence
  C4m#19-5th4w-NN6-68
GGCLHPWLPIRSRHFCSR

SEQ ID NO: 116 - protein, 18 aa, Artificial Sequence
  C4m3127-4th-NNS6-28
GGCLHPFLPIFSSHFCAL

SEQ ID NO: 117 - protein, 18 aa, Artificial Sequence
  C4m#19-5th4w-NN6-7
GGCRHPFLPIWSWHFCPF

SEQ ID NO: 118 - protein, 18 aa, Artificial Sequence
  C4m#19-5th4w-NN6-85
GGCWHPFLPIFSVHFCGC

SEQ ID NO: 119 - protein, 18 aa, Artificial Sequence
  C4m#19-5th2w-NNS6-71
GGCRHPYLPIASPHFCPG

SEQ ID NO: 120 - protein, 18 aa, Artificial Sequence
  C4m3127-4th-NNS6-90
GGCKHPVLPIVSLHFCPW

SEQ ID NO: 121 - protein, 18 aa, Artificial Sequence
  C4m#19-5th4w-NN6-37
GGCLHPFLPISSWHFCGR

SEQ ID NO: 122 - protein, 18 aa, Artificial Sequence
  C4m#19-5th2w-NNS6-94
GGCFHPYLPISSVHFCGR

SEQ ID NO: 123 - protein, 18 aa, Artificial Sequence
  C4m#19-5th4w-NN6-51
GGCWHPYLPIVSWHFCSR

SEQ ID NO: 124 - protein, 18 aa, Artificial Sequence
  C4m#19-5th4w-NN6-11
GGCRHPFLPIWSHHFCVC

SEQ ID NO: 125 - protein, 18 aa, Artificial Sequence
  C4m#19-5th4w-NN6-87
GGCLHPVLPIRSFHFCWR

SEQ ID NO: 126 - protein, 18 aa, Artificial Sequence
  C4m3127-4th-NNS6-87
GGCRHPWLPIVSWHFCSR

SEQ ID NO: 127 - protein, 18 aa, Artificial Sequence
  C4m#19-5th4w-NN6-90
GGCRHPWLPIVSYHFCSS

SEQ ID NO: 128 - protein, 18 aa, Artificial Sequence
  C4m#19-5th2w-NNS6-25
GGCKHPFLPISSHHFCPY

SEQ ID NO: 129 - protein, 18 aa, Artificial Sequence
  C4m3127-4th-NNS6-83
GGCRHPFLPIFSKHFCEL

SEQ ID NO: 130 - protein, 18 aa, Artificial Sequence
  C4m3127-4th-NNS6-17
GGCRHPVLPIVSLHFCPG

SEQ ID NO: 131 - protein, 18 aa, Artificial Sequence
  C4m#19-5th2w-NNS6-12
GGCWHPYLPIRSVHFCGR

SEQ ID NO: 132 - protein, 18 aa, Artificial Sequence
  C4m3127-4th-NNS6-72
GGCVHPYLPISSIHFCSM

SEQ ID NO: 133 - protein, 18 aa, Artificial Sequence
  C4m#19-5th2w-NNS6-90
GGCRHPFLPIVSFHFCPF

SEQ ID NO: 134 - protein, 18 aa, Artificial Sequence
  C4m#19-5th4w-NN6-86
GGCAHPVLPIRSLHFCPH

SEQ ID NO: 135 - protein, 18 aa, Artificial Sequence
  C4m#19-5th4w-NN6-58
GGCRHPFLPISSIHFCCI

SEQ ID NO: 136 - protein, 18 aa, Artificial Sequence
  C4m#19-5th2w-NNS6-3
GGCAHPFLPIFSPHFCPF

SEQ ID NO: 137 - protein, 18 aa, Artificial Sequence
  C4m#19-5th4w-NN6-2
GGCWHPHLPIVSSHFCLF

SEQ ID NO: 138 - protein, 18 aa, Artificial Sequence
  C4m#19-5th4w-NN6-71
GGCPHPWLPIASVHFCPF

SEQ ID NO: 139 - protein, 18 aa, Artificial Sequence
  C4m#19-5th4w-NN6-62
GGCQHPYLPIWSFHFCPF

SEQ ID NO: 140 - protein, 18 aa, Artificial Sequence
  C4m#19-5th4w-NN6-30
GGCWHPFLPIMSFHFCPY

SEQ ID NO: 141 - protein, 18 aa, Artificial Sequence
  C4m#19-5th4w-NN6-38
GGCSHPFLPIFSLHFCPV

SEQ ID NO: 142 - protein, 18 aa, Artificial Sequence
  C4m#19-5th2w-NNS6-8
GGCRHPFLPIFSLHFCAR

SEQ ID NO: 143 - protein, 18 aa, Artificial Sequence
  C4m3127-4th-NNS6-16
GGCWHPYLPIFSVHFCPR

SEQ ID NO: 144 - protein, 18 aa, Artificial Sequence
  C4m#19-5th4w-NN6-63
GGCWHPYLPILSRHFCQA

SEQ ID NO: 145 - protein, 18 aa, Artificial Sequence
  C4m#19-5th4w-NN6-14
GGCWHPFLPIRSVHFCCR

SEQ ID NO: 146 - protein, 18 aa, Artificial Sequence
  C4m#19-5th4w-NN6-1
GGCRHPYLPIFSAHFCRS

SEQ ID NO: 147 - protein, 18 aa, Artificial Sequence
  C4m#19-5th4w-NN6-6
GGCMHPFLPIKSSHFCRK

SEQ ID NO: 148 - protein, 18 aa, Artificial Sequence
  C4m#19-5th2w-NNS6-51
GGCRHPFLPIVSLHFCPF

SEQ ID NO: 149 - protein, 18 aa, Artificial Sequence
  C4m#19-5th4w-NN6-45
GGCRHPWLPIWSVHFCGV

SEQ ID NO: 150 - protein, 18 aa, Artificial Sequence
  C4m3127-4th-NNS6-12
GGCSHPFLPIRSRHFCPF

SEQ ID NO: 151 - protein, 18 aa, Artificial Sequence
  C4m#19-5th2w-NNS6-75
GGCWHPWLPIKSPHFCAL

SEQ ID NO: 152 - protein, 18 aa, Artificial Sequence
  C4m#19-5th4w-NN6-74
GGCFHPFLPIYSWHFCAR

SEQ ID NO: 153 - protein, 18 aa, Artificial Sequence
  C4m#19-5th4w-NN6-5-1
GGCWHPYLPIQSLHFCPF

SEQ ID NO: 154 - protein, 18 aa, Artificial Sequence
  C4m#19-5th4w-NN6-5-3
GGCWHPFLPILSLHFCGW

SEQ ID NO: 155 - protein, 18 aa, Artificial Sequence
  C4m#19-5th4w-NN6-46-1
GGCVHPALPIWSFHFCPS

SEQ ID NO: 156 - protein, 18 aa, Artificial Sequence
  C4m#19-5th4w-NN6-64
GGCWHPVLPIRSVHFCCR

SEQ ID NO: 157 - protein, 18 aa, Artificial Sequence
  C4m3127-4th-NNS6-48
GGCFHPWLPIASWHFCGR

SEQ ID NO: 158 - protein, 18 aa, Artificial Sequence
  C4m3127-4th-NNS6-64
GGCLHPYLPIVSSHFCPF

SEQ ID NO: 159 - protein, 18 aa, Artificial Sequence
  C4m3127-4th-NNS6-80
GGCGHPFLPIFSLHFCPR

SEQ ID NO: 160 - protein, 18 aa, Artificial Sequence
  C4m3127-4th-NNS6-79
GGCLHPFLPIRSVHFCLR

SEQ ID NO: 161 - protein, 18 aa, Artificial Sequence
  C4m3127-4th-NNS6-2
GGCWHPSLPIYSPHFCPL

SEQ ID NO: 162 - protein, 18 aa, Artificial Sequence
  C4m#19-5th4w-NN6-65
GGCWHPFLPILSLHFCSR

SEQ ID NO: 163 - protein, 18 aa, Artificial Sequence
  C4m#19-5th4w-NN6-83
GGCLHPLLPILSVHFCPS

SEQ ID NO: 164 - protein, 18 aa, Artificial Sequence
  C4m3127-4th-NNS6-60
GGCWHPFLPISSWHFCGL

SEQ ID NO: 165 - protein, 18 aa, Artificial Sequence
  C4m#19-5th2w-NNS6-53
GGCLHPWLPIRSFHFCGA

SEQ ID NO: 166 - protein, 18 aa, Artificial Sequence
  C4m#19-5th2w-NNS6-45
GGCRHPFLPIWSVHFCWR

SEQ ID NO: 167 - protein, 18 aa, Artificial Sequence
  C4m3127-4th-NNS6-3
GGCSHPFLPIWSVHFCGQ

SEQ ID NO: 168 - protein, 18 aa, Artificial Sequence
  C4m#19-5th2w-NNS6-6
GGCWHPYLPILSLHFCQR

SEQ ID NO: 169 - protein, 18 aa, Artificial Sequence
  C4m#19-5th2w-NNS6-27
GGCFHPFLPIRSCHFCAR

SEQ ID NO: 170 - protein, 18 aa, Artificial Sequence
  C4m#19-5th2w-NNS6-37
GGCIHPFLPIWSIHFCSR

SEQ ID NO: 171 - protein, 18 aa, Artificial Sequence
  C4m#19-5th2w-NNS6-33
GGCRHPFLPIWSFHFCWG

SEQ ID NO: 172 - protein, 18 aa, Artificial Sequence
  C4m#19-5th2w-NNS6-79
GGCRHPFLPIVSRHFCVA

SEQ ID NO: 173 - protein, 18 aa, Artificial Sequence
  C4m3127-4th-NNS6-85
GGCGHPFLPIFSSHFCPL

SEQ ID NO: 174 - protein, 18 aa, Artificial Sequence
  C4m#19-5th2w-NNS6-30
GGCWHPFLPILSWHFCGR

SEQ ID NO: 175 - protein, 18 aa, Artificial Sequence
  C4m#19-5th4w-NN6-89
GGCMHPFLPIISQHFCAF

SEQ ID NO: 176 - protein, 18 aa, Artificial Sequence
  C4m#19-5th2w-NNS6-86
GGCFHPYLPIWSLHFCRS

SEQ ID NO: 177 - protein, 18 aa, Artificial Sequence
  C4m3127-4th-NNS6-30
GGCWHPCLPILSPHFCPR

SEQ ID NO: 178 - protein, 18 aa, Artificial Sequence
  C4m3127-4th-NNS6-26
GGCAHPALPIWSCHFCPF

SEQ ID NO: 179 - protein, 18 aa, Artificial Sequence
  C4m#19-5th2w-NNS6-74
GGCMHPFLPIRSWHFCSR

SEQ ID NO: 180 - protein, 18 aa, Artificial Sequence
  C4m3127-4th-NNS6-89
GGCWHPFLPIFSAHFCMR

SEQ ID NO: 181 - protein, 18 aa, Artificial Sequence
  C4m#19-5th2w-NNS6-84
GGCWHPFLPIVSFHFCPF

SEQ ID NO: 182 - protein, 18 aa, Artificial Sequence
  C4m#19-5th2w-NNS6-28
GGCAHPYLPIRSVHFCPC

SEQ ID NO: 183 - protein, 18 aa, Artificial Sequence
  C4m#19-5th2w-NNS6-4
GGCFHPWLPISSLHFCPF

SEQ ID NO: 184 - protein, 18 aa, Artificial Sequence
  C4m#19-5th2w-NNS6-46
GGCFHPFLPIFSYHFCGL

SEQ ID NO: 185 - protein, 18 aa, Artificial Sequence
  C4m#19-5th4w-NN6-61
GGCPHPMLPIFSVHFCPY

SEQ ID NO: 186 - protein, 18 aa, Artificial Sequence
  C4m3127-4th-NNS6-94
GGCRHPVLPIWSSHFCPW

SEQ ID NO: 187 - protein, 18 aa, Artificial Sequence
  C4m#19-5th2w-NNS6-26
GGCLHPFLPIVSIHFCSA

SEQ ID NO: 188 - protein, 18 aa, Artificial Sequence
  C4m#19-5th4w-NN6-36
GGCRHPYLPIWSAHFCCR

SEQ ID NO: 189 - protein, 18 aa, Artificial Sequence
  C4m#19-5th4w-NN6-75
GGCWHPFLPIKSVHFCCA

SEQ ID NO: 190 - protein, 18 aa, Artificial Sequence
  C4m#19-5th2w-NNS6-70
GGCRHPFLPIVSWHFCAA

SEQ ID NO: 191 - protein, 18 aa, Artificial Sequence
  C4m#19-5th2w-NNS6-34
GGCCHPFLPIYSVHFCAS

SEQ ID NO: 192 - protein, 18 aa, Artificial Sequence
  C4m#19-5th4w-NN6-94
GGCLHPFLPIYSLHFCPC

SEQ ID NO: 193 - protein, 18 aa, Artificial Sequence
  C4m3127-4th-NNS6-66
GGCAHPHLPIRSVHFCSF

SEQ ID NO: 194 - protein, 18 aa, Artificial Sequence
  C4m#19-5th2w-NNS6-43
GGCRHPFLPIWSSHFCAA

SEQ ID NO: 195 - protein, 18 aa, Artificial Sequence
  C4m3127-4th-NNS6-7
GGCRHPFLPIRSPHFCGS

SEQ ID NO: 196 - protein, 18 aa, Artificial Sequence
  C4m#19-5th4w-NN6-72
GGCWHPWLPIVSVHFCGC

SEQ ID NO: 197 - protein, 18 aa, Artificial Sequence
  C4m3127-4th-NNS6-70
GGCSHPYLPIHSRHFCLS

SEQ ID NO: 198 - protein, 18 aa, Artificial Sequence
  C4m#19-5th2w-NNS6-68
GGCLHPWLPIVSCHFCPR

SEQ ID NO: 199 - protein, 18 aa, Artificial Sequence
  C4m#19-5th2w-NNS6-87
GGCLHPYLPIFSVHFCAL

SEQ ID NO: 200 - protein, 18 aa, Artificial Sequence
  C4m#19-5th2w-NNS6-66
GGCRHPFLPIFSVHFCPF

SEQ ID NO: 201 - protein, 18 aa, Artificial Sequence
  C4m3127-4th-NNS6-20
GGCLHPFLPILSLHFCPF

SEQ ID NO: 202 - protein, 18 aa, Artificial Sequence
  C4m#19-5th2w-NNS6-61
GGCCHPWLPIRSVHFCPF

SEQ ID NO: 203 - protein, 18 aa, Artificial Sequence
  C4m3127-4th-NNS6-19
GGCMHPSLPIWSWHFCPH

SEQ ID NO: 204 - protein, 18 aa, Artificial Sequence
  C4m#19-5th4w-NN6-40
GGCFHPFLPIRSHHFCML

SEQ ID NO: 205 - protein, 18 aa, Artificial Sequence
  C4m#19-5th4w-NN6-49
GGCMHPYLPIRSFHFCSC

SEQ ID NO: 206 - protein, 18 aa, Artificial Sequence
  C4m#19-5th4w-NN6-80
GGCRHPFLPIFSWHFCAV

SEQ ID NO: 207 - protein, 18 aa, Artificial Sequence
  C4m#19-5th2w-NNS6-80
GGCLHPFLPIVSWHFCPC

SEQ ID NO: 208 - protein, 18 aa, Artificial Sequence
  C4m3127-4th-NNS6-37
GGCWHPVLPIRSIHFCGC

SEQ ID NO: 209 - protein, 18 aa, Artificial Sequence
  C4m#19-5th2w-NNS6-93
GGCFHPFLPIQSRHFCCR

SEQ ID NO: 210 - protein, 18 aa, Artificial Sequence
  C4m3127-4th-NNS6-95
GGCWHPVLPIRSGHFCSR

SEQ ID NO: 211 - protein, 18 aa, Artificial Sequence
  C4m#19-5th2w-NNS6-41
GGCWHPVLPIRSDHFCCR